European Patent Application EP 4 678 662 A1, published January 14, 2026. Title: 免疫グロブリン. Applicant: 国立大学法人　東京大学. Application JP, filed March 4, 2024. The sequence listing filed with the application follows.

SEQUENCE LISTING (14 sequences)

SEQ ID NO: 1 - protein, 504 aa, synthetic construct
EVQLQQSGSELVKSGASVKLSCTVSGFNFTDYYIHWVRQRTEQGLEWIGRIDPENDETTYAPKFQGKATMTADTSSNTAYLQLTSLTSEDTAVYYCARSTVLDYWGHGTTLTVSSESARNPTIYPLTLPRALSSDPVIIGCLIHDYFPSGTMNVTWGKSGKDITTVNFPPALASGGGYTMSSQLTLPAVECPEGESVKCSVQHDSNAVQELDVKCSGPPPPCPPCPPSCHPSLSLQRPALEDLLLGSDASLTCTLNGLRNPEGAVFTWEPSTGKDAVQKKAVQNSCGCYSVSSVLPGCAERWNSGASFKCTVTHPESDTLTGTIAKITVNTFPPQVHLLPPPSEELALNELVSLTCLVRAFNPKEVLVRWLHGNEELSPESYLVFEPLKEPGEGATTYLVTSVLRVSAELWKQGDQYSCMVGHEALPMNFTQKTIDRLSGKNSEGQIPLGGDLAPQMLRELQETNAALQDVRELLRQQVKEITFLKNTVMECDACGMQPARTPG

SEQ ID NO: 2 - DNA, 1572 bp, synthetic construct
  source 1..1572: mol_type = other DNA
atgaaatgcagctggatcatcttcttcctgatggcagtggttacaggggtcaattcagaggttcagctgcagcagtctgggtcagagcttgtgaagtctggggcctcagtcaagttgtcctgcacagtttctgggttcaactttacagactactatatacactgggtgaggcagaggactgaacagggcctggaatggattggaaggattgatcctgagaatgatgaaactacatatgccccgaaattccagggcaaggccactatgacagcagacacatcttccaacacagcctacctgcagctcaccagcctgacatctgaagacactgccgtctattactgtgctagatctacggtccttgactactggggccacggcaccactctcacagtctcctcagagtctgcgagaaatcccaccatctacccactgacactcccacgagctctgtcaagtgacccagtgataatcggctgcctgattcacgattacttcccttccggcacgatgaatgtgacctggggaaagagtgggaaggatataaccaccgtaaacttcccacctgccctggcctctgggggagggtacaccatgagcagccagttgaccctgccagctgtcgagtgcccagaaggagaatccgtgaaatgttccgtgcaacatgactctaacgccgtccaagaattggatgtgaagtgctctggtcctcctcctccttgtcctccttgtcctccttcctgccatcccagcctgtcactgcagcggccagctcttgaggacctgctcctgggttcagatgccagcctcacatgtactctgaatggcctgagaaatcctgagggagctgtcttcacctgggagccctccactgggaaggatgcagtgcagaagaaagctgtgcagaattcctgcggctgctacagtgtgtccagcgtcctgcctggctgtgctgagcgctggaacagtggcgcatcattcaagtgcacagttacccatcctgagtctgacaccttaactggcacaattgccaaaatcacagtgaacaccttcccaccccaggtccacctgctaccgccgccgtcggaggagctggccctgaatgagctcgtgtccctgacatgcctggtgcgagctttcaaccctaaagaagtgctggtgcgatggctgcatggaaatgaggagctgtccccagaaagctacctagtgtttgagcccctaaaggagccaggcgagggagccaccacctacctggtgacaagcgtgttgcgtgtatcagctgaactctggaaacagggtgaccagtactcctgcatggtgggccacgaggccttgcccatgaacttcacccagaagaccatcgaccgtctgtcgggtaaaaattcagagggccagatcccgctgggtggagacctggccccacagatgctgcgagaacttcaggagactaatgcggcgctgcaagacgtgagagagctgttgcgacagcaggtcaaggagatcaccttcctgaagaatacggtgatggaatgtgatgcttgcggaatgcagcccgcacgcactccaggctga

SEQ ID NO: 3 - protein, 131 aa, synthetic construct
MKLPVRLLVLMFWIPGFSSDVLMTQSPASLSVSLGDRATISCRASQSIVHTNGNTYLEWYLQKPGQSPKLLIYKVSNRFSGVPDRFSGSGSGTDFILKISRVEAEDLGVYYCFQGSHVPPTFGGGTKLEVK

SEQ ID NO: 4 - protein, 26 aa, synthetic construct
SSADDAKKDAAKKDDAKKDDAKKDAS

SEQ ID NO: 5 - protein, 26 aa, synthetic construct
SSADDAAADAAAADDAAADDAAADAS

SEQ ID NO: 6 - protein, 19 aa, synthetic construct
MKCSWIIFFLMAVVTGVNS

SEQ ID NO: 7 - protein, 18 aa, synthetic construct
PTNVSVSVIMSEGDGICY

SEQ ID NO: 8 - protein, 504 aa, synthetic construct; identical to SEQ ID NO: 1

SEQ ID NO: 9 - protein, 548 aa, synthetic construct
EVQLQQSGSELVKSGASVKLSCTVSGFNFTDYYIHWVRQRTEQGLEWIGRIDPENDETTYAPKFQGKATMTADTSSNTAYLQLTSLTSEDTAVYYCARSTVLDYWGHGTTLTVSSESARNPTIYPLTLPRALSSDPVIIGCLIHDYFPSGTMNVTWGKSGKDITTVNFPPALASGGGYTMSSQLTLPAVECPEGESVKCSVQHDSNAVQELDVKCSGPPPPCPPCPPSCHPSLSLQRPALEDLLLGSDASLTCTLNGLRNPEGAVFTWEPSTGKDAVQKKAVQNSCGCYSVSSVLPGCAERWNSGASFKCTVTHPESDTLTGTIAKITVNTFPPQVHLLPPPSEELALNELVSLTCLVRAFNPKEVLVRWLHGNEELSPESYLVFEPLKEPGEGATTYLVTSVLRVSAELWKQGDQYSCMVGHEALPMNFTQKTIDRLSGKPTNVSVSVIMSEGDGICYSSADDAKKDAAAADDKKADDAKKDASNSEGQIPLGGDLAPQMLRELQETNAALQDVRELLRQQVKEITFLKNTVMECDACGMQPARTPG

SEQ ID NO: 10 - protein, 522 aa, synthetic construct
EVQLQQSGSELVKSGASVKLSCTVSGFNFTDYYIHWVRQRTEQGLEWIGRIDPENDETTYAPKFQGKATMTADTSSNTAYLQLTSLTSEDTAVYYCARSTVLDYWGHGTTLTVSSESARNPTIYPLTLPRALSSDPVIIGCLIHDYFPSGTMNVTWGKSGKDITTVNFPPALASGGGYTMSSQLTLPAVECPEGESVKCSVQHDSNAVQELDVKCSGPPPPCPPCPPSCHPSLSLQRPALEDLLLGSDASLTCTLNGLRNPEGAVFTWEPSTGKDAVQKKAVQNSCGCYSVSSVLPGCAERWNSGASFKCTVTHPESDTLTGTIAKITVNTFPPQVHLLPPPSEELALNELVSLTCLVRAFNPKEVLVRWLHGNEELSPESYLVFEPLKEPGEGATTYLVTSVLRVSAELWKQGDQYSCMVGHEALPMNFTQKTIDRLSGKPTNVSVSVIMSEGDGICYNSEGQIPLGGDLAPQMLRELQETNAALQDVRELLRQQVKEITFLKNTVMECDACGMQPARTPG

SEQ ID NO: 11 - DNA, 1704 bp, synthetic construct
  source 1..1704: mol_type = other DNA
atgaaatgcagctggatcatcttcttcctgatggcagtggttacaggggtcaattcagaggttcagctgcagcagtctgggtcagagcttgtgaagtctggggcctcagtcaagttgtcctgcacagtttctgggttcaactttacagactactatatacactgggtgaggcagaggactgaacagggcctggaatggattggaaggattgatcctgagaatgatgaaactacatatgccccgaaattccagggcaaggccactatgacagcagacacatcttccaacacagcctacctgcagctcaccagcctgacatctgaagacactgccgtctattactgtgctagatctacggtccttgactactggggccacggcaccactctcacagtctcctcagagtctgcgagaaatcccaccatctacccactgacactcccacgagctctgtcaagtgacccagtgataatcggctgcctgattcacgattacttcccttccggcacgatgaatgtgacctggggaaagagtgggaaggatataaccaccgtaaacttcccacctgccctggcctctgggggagggtacaccatgagcagccagttgaccctgccagctgtcgagtgcccagaaggagaatccgtgaaatgttccgtgcaacatgactctaacgccgtccaagaattggatgtgaagtgctctggtcctcctcctccttgtcctccttgtcctccttcctgccatcccagcctgtcactgcagcggccagctcttgaggacctgctcctgggttcagatgccagcctcacatgtactctgaatggcctgagaaatcctgagggagctgtcttcacctgggagccctccactgggaaggatgcagtgcagaagaaagctgtgcagaattcctgcggctgctacagtgtgtccagcgtcctgcctggctgtgctgagcgctggaacagtggcgcatcattcaagtgcacagttacccatcctgagtctgacaccttaactggcacaattgccaaaatcacagtgaacaccttcccaccccaggtccacctgctaccgccgccgtcggaggagctggccctgaatgagctcgtgtccctgacatgcctggtgcgagctttcaaccctaaagaagtgctggtgcgatggctgcatggaaatgaggagctgtccccagaaagctacctagtgtttgagcccctaaaggagccaggcgagggagccaccacctacctggtgacaagcgtgttgcgtgtatcagctgaactctggaaacagggtgaccagtactcctgcatggtgggccacgaggccttgcccatgaacttcacccagaagaccatcgaccgtctgtcgggtaaacccaccaatgtcagcgtgtctgtgatcatgtcagagggagatggcatctgctactcctccgctgacgatgccgctgctgatgctgccgccgccgatgatgctgctgctgacgacgccgctgctgacgcttccaactccgagggccagatcccgctgggtggagacctggccccacagatgctgcgagaacttcaggagactaatgcggcgctgcaagacgtgagagagctgttgcgacagcaggtcaaggagatcaccttcctgaagaatacggtgatggaatgtgatgcttgcggaatgcagcccgcacgcactccaggctga

SEQ ID NO: 12 - DNA, 1704 bp, synthetic construct
  source 1..1704: mol_type = other DNA
atgaaatgcagctggatcatcttcttcctgatggcagtggttacaggggtcaattcagaggttcagctgcagcagtctgggtcagagcttgtgaagtctggggcctcagtcaagttgtcctgcacagtttctgggttcaactttacagactactatatacactgggtgaggcagaggactgaacagggcctggaatggattggaaggattgatcctgagaatgatgaaactacatatgccccgaaattccagggcaaggccactatgacagcagacacatcttccaacacagcctacctgcagctcaccagcctgacatctgaagacactgccgtctattactgtgctagatctacggtccttgactactggggccacggcaccactctcacagtctcctcagagtctgcgagaaatcccaccatctacccactgacactcccacgagctctgtcaagtgacccagtgataatcggctgcctgattcacgattacttcccttccggcacgatgaatgtgacctggggaaagagtgggaaggatataaccaccgtaaacttcccacctgccctggcctctgggggagggtacaccatgagcagccagttgaccctgccagctgtcgagtgcccagaaggagaatccgtgaaatgttccgtgcaacatgactctaacgccgtccaagaattggatgtgaagtgctctggtcctcctcctccttgtcctccttgtcctccttcctgccatcccagcctgtcactgcagcggccagctcttgaggacctgctcctgggttcagatgccagcctcacatgtactctgaatggcctgagaaatcctgagggagctgtcttcacctgggagccctccactgggaaggatgcagtgcagaagaaagctgtgcagaattcctgcggctgctacagtgtgtccagcgtcctgcctggctgtgctgagcgctggaacagtggcgcatcattcaagtgcacagttacccatcctgagtctgacaccttaactggcacaattgccaaaatcacagtgaacaccttcccaccccaggtccacctgctaccgccgccgtcggaggagctggccctgaatgagctcgtgtccctgacatgcctggtgcgagctttcaaccctaaagaagtgctggtgcgatggctgcatggaaatgaggagctgtccccagaaagctacctagtgtttgagcccctaaaggagccaggcgagggagccaccacctacctggtgacaagcgtgttgcgtgtatcagctgaactctggaaacagggtgaccagtactcctgcatggtgggccacgaggccttgcccatgaacttcacccagaagaccatcgaccgtctgtcgggtaaacccaccaatgtcagcgtgtctgtgatcatgtcagagggagatggcatctgctacagctcggcagacgatgccaagaaagatgcagccaagaaagacgatgccaagaaagacgacgccaagaaagacgcttccaattcagagggccagatcccgctgggtggagacctggccccacagatgctgcgagaacttcaggagactaatgcggcgctgcaagacgtgagagagctgttgcgacagcaggtcaaggagatcaccttcctgaagaatacggtgatggaatgtgatgcttgcggaatgcagcccgcacgcactccaggctga

SEQ ID NO: 13 - DNA, 1626 bp, synthetic construct
  source 1..1626: mol_type = other DNA
atgaaatgcagctggatcatcttcttcctgatggcagtggttacaggggtcaattcagaggttcagctgcagcagtctgggtcagagcttgtgaagtctggggcctcagtcaagttgtcctgcacagtttctgggttcaactttacagactactatatacactgggtgaggcagaggactgaacagggcctggaatggattggaaggattgatcctgagaatgatgaaactacatatgccccgaaattccagggcaaggccactatgacagcagacacatcttccaacacagcctacctgcagctcaccagcctgacatctgaagacactgccgtctattactgtgctagatctacggtccttgactactggggccacggcaccactctcacagtctcctcagagtctgcgagaaatcccaccatctacccactgacactcccacgagctctgtcaagtgacccagtgataatcggctgcctgattcacgattacttcccttccggcacgatgaatgtgacctggggaaagagtgggaaggatataaccaccgtaaacttcccacctgccctggcctctgggggagggtacaccatgagcagccagttgaccctgccagctgtcgagtgcccagaaggagaatccgtgaaatgttccgtgcaacatgactctaacgccgtccaagaattggatgtgaagtgctctggtcctcctcctccttgtcctccttgtcctccttcctgccatcccagcctgtcactgcagcggccagctcttgaggacctgctcctgggttcagatgccagcctcacatgtactctgaatggcctgagaaatcctgagggagctgtcttcacctgggagccctccactgggaaggatgcagtgcagaagaaagctgtgcagaattcctgcggctgctacagtgtgtccagcgtcctgcctggctgtgctgagcgctggaacagtggcgcatcattcaagtgcacagttacccatcctgagtctgacaccttaactggcacaattgccaaaatcacagtgaacaccttcccaccccaggtccacctgctaccgccgccgtcggaggagctggccctgaatgagctcgtgtccctgacatgcctggtgcgagctttcaaccctaaagaagtgctggtgcgatggctgcatggaaatgaggagctgtccccagaaagctacctagtgtttgagcccctaaaggagccaggcgagggagccaccacctacctggtgacaagcgtgttgcgtgtatcagctgaactctggaaacagggtgaccagtactcctgcatggtgggccacgaggccttgcccatgaacttcacccagaagaccatcgaccgtctgtcgggtaaacccaccaatgtcagcgtgtctgtgatcatgtcagagggagatggcatctgctacaattcagagggccagatcccgctgggtggagacctggccccacagatgctgcgagaacttcaggagactaatgcggcgctgcaagacgtgagagagctgttgcgacagcaggtcaaggagatcaccttcctgaagaatacggtgatggaatgtgatgcttgcggaatgcagcccgcacgcactccaggctga

SEQ ID NO: 14 - DNA, 1572 bp, synthetic construct; identical to SEQ ID NO: 2
  source 1..1572: mol_type = other DNA